European Patent Application EP 4 570 900 A1, published June 18, 2025. Title: 一株植物乳杆菌及其应用. Applicant: 成都倍特生物制药有限公司. The sequence listing filed with the application follows.

SEQUENCE LISTING (4 sequences)

SEQ ID NO: 1 - DNA, 1439 bp, synthetic construct
  source 1..1439: mol_type = other DNA
tgcaagtcgaacgaactctggtattgattggtgcttgcatcatgatttacatttgagtgagtggcgaactggtgagtaacacgtgggaaacctgcccagaagcgggggataacacctggaaacagatgctaataccgcataacaacttggaccgcatggtccgagcttgaaagatggcttcggctatcacttttggatggtcccgcggcgtattagctagatggtggggtaacggctcaccatggcaatgatacgtagccgacctgagagggtaatcggccacattgggactgagacacggcccaaactcctacgggaggcagcagtagggaatcttccacaatggacgaaagtctgatggagcaacgccgcgtgagtgaagaagggtttcggctcgtaaaactctgttgttaaagaagaacatatctgagagtaactgttcaggtattgacggtatttaaccagaaagccacggctaactacgtgccagcagccgcggtaatacgtaggtggcaagcgttgtccggatttattgggcgtaaagcgagcgcaggcggttttttaagtctgatgtgaaagccttcggctcaaccgaagaagtgcatcggaaactgggaaacttgagtgcagaagaggacagtggaactccatgtgtagcggtgaaatgcgtagatatatggaagaacaccagtggcgaaggcggctgtctggtctgtaactgacgctgaggctcgaaagtatgggtagcaaacaggattagataccctggtagtccataccgtaaacgatgaatgctaagtgttggagggtttccgcccttcagtgctgcagctaacgcattaagcattccgcctggggagtacggccgcaaggctgaaactcaaaggaattgacgggggcccgcacaagcggtggagcatgtggtttaattcgaagctacgcgaagaaccttaccaggtcttgacatactatgcaaatctaagagattagacgttcccttcggggacatggatacaggtggtgcatggttgtcgtcagctcgtgtcgtgagatgttgggttaagtcccgcaacgagcgcaacccttattatcagttgccagcattaagttgggcactctggtgagactgccggtgacaaaccggaggaaggtggggatgacgtcaaatcatcatgccccttatgacctgggctacacacgtgctacaatggatggtacaacgagttgcgaactcgcgagagtaagctaatctcttaaagccattctcagttcggattgtaggctgcaactcgcctacatgaagtcggaatcgctagtaatcgcggatcagcatgccgcggtgaatacgttcccgggccttgtacacaccgcccgtcacaccatgagagtttgtaacacccaaagtcggtggggtaaccttttaggaaccagccgcctaa

SEQ ID NO: 2 - DNA, 1439 bp, synthetic construct
  source 1..1439: mol_type = other DNA
cagtcgagcgagcttgcctagatgaatttggtgcttgcaccagatgaaactagatacaagcgagcggcggacgggtgagtaacacgtgggtaacctgcccaagagactgggataacacctggaaacagatgctaataccggataacaacactagacgcatgtctagagtttaaaagatggttctgctatcactcttggatggacctgcggtgcattagctagttggtaaggcaacggcttaccaaggcaatgatgcatagccgagttgagagactgatcggccacattgggactgagacacggcccaaactcctacgggaggcagcagtagggaatcttccacaatggacgcaagtctgatggagcaacgccgcgtgagtgaagaagggtttcggctcgtaaagctctgttggtagtgaagaaagatagaggtagtaactggcctttatttgacggtaattacttagaaagtcacggctaactacgtgccagcagccgcggtaatacgtaggtggcaagcgttgtccggatttattgggcgtaaagcgagtgcaggcggttcaataagtctgatgtgaaagccttcggctcaaccggagaattgcatcagaaactgctgaacttgagtgcagaagaggagagtggaactccatgtgtagcggtggaatgcgtagatatatggaagaacaccagtggcgaaggcggctctctggtctgcaactgacgctgaggctcgaaagcatgggtagcgaacaggattagataccctggtagtccatgccgtaaacgatgagtgctaagtgttgggaggtttccgcctctcagtgctgcagctaacgcattaagcactccgcctggggagtacgaccgcaaggttgaaactcaaaggaattgacgggggcccgcacaagcggtggagcatgtggtttaattcgaagcaacgcgaagaaccttaccaggtcttgacatccagtgcaaacctaagagattaggagttcccttcggggacgctgagacaggtggtgcatggctgtcgtcagctcgtgtcgtgagatgttgggttaagtcccgcaacgagcgcaacccttgtcattagttgccatcattaagttgggcactctaatgagactgccggtgacaaaccggaggaaggtggggatgacgtcaagtcatcatgccccttatgacctgggctacacacgtgctacaatggacggtacaacgagaagcgaacctgcgaaggcaagcggatctctgaaagccgttctcagttcggactgtaggctgcaactcgcctacacgaagctggaatcgctagtaatcgcggatcagcacgccgcggtgaatacgttcccgggccttgtacacaccgcccgtcacaccatgagagtctgtaacacccaaagccggtgggataacctttataggagtcagccgtc

SEQ ID NO: 3 - DNA, 1425 bp, synthetic construct
  source 1..1425: mol_type = other DNA
gtcgagcgagcttgcctatagaaattcttcggaatggacatagatacaagctagcggcggatgggtgagtaacgcgtgggtaacctgcccttaagtctgggataccatttggaaacagatgctaataccggataaaagctactttcgcatgaaagaagtttaaaaggcggcgtaagctgtcgctaaaggatggacctgcgatgcattagctagttggtaaggtaacggcttaccaaggcgatgatgcatagccgagttgagagactgatcggccacattgggactgagacacggcccaaactcctacgggaggcagcagtagggaatcttccacaatggacgaaagtctgatggagcaacgccgcgtgagtgaagaaggttttcggatcgtaaagctctgttgttggtgaagaaggatagaggtagtaactggcctttatttgacggtaatcaaccagaaagtcacggctaactacgtgccagcagccgcggtaatacgtaggtggcaagcgttgtccggatttattgggcgtaaagcgagcgcaggcggattgataagtctgatgtgaaagccttcggctcaaccgaagaactgcatcagaaactgtcaatcttgagtgcagaagaggagagtggaactccatgtgtagcggtggaatgcgtagatatatggaagaacaccagtggcgaaggcggctctctggtctgtaactgacgctgaggctcgaaagcatgggtagcgaacaggattagataccctggtagtccatgccgtaaacgatgagtgctaagtgttgggaggtttccgcctctcagtgctgcagctaacgcattaagcactccgcctggggagtacgaccgcaaggttgaaactcaaaggaattgacgggggcccgcacaagcggtggagcatgtggtttaattcgaagcaacgcgaagaaccttaccaggtcttgacatcctttgaccacctaagagattaggttttcccttcggggacaaagagacaggtggtgcatggctgtcgtcagctcgtgtcgtgagatgttgggttaagtcccgcaacgagcgcaacccttgttaatagttgccagcattaagttgggcactctattgagactgccggtgacaaaccggaggaaggtggggatgacgtcaagtcatcatgccccttatgacctgggctacacacgtgctacaatgggcagtacaacgagaagcgaacctgtgaaggcaagcggatctcttaaagctgttctcagttcggactgtaggctgcaactcgcctacacgaagctggaatcgctagtaatcgcggatcagcacgccgcggtgaatacgttcccgggccttgtacacaccgcccgtcacaccatgagagtttgtaacacccaaagtcggtgaggtaacctttggagccagccg

SEQ ID NO: 4 - DNA, 1433 bp, synthetic construct
  source 1..1433: mol_type = other DNA
ctgcaagtcgagcgagcggaactaacagatttacttcggtaatgacgttaggaaagcgagcggcggatgggtgagtaacacgtggggaacctgccccatagtctgggataccacttggaaacaggtgctaataccggataagaaagcagatcgcatgatcagcttttaaaaggcggcgtaagctgtcgctatgggatggccccgcggtgcattagctagttggtaaggtaaaggcttaccaaggcgatgatgcatagccgagttgagagactgatcggccacattgggactgagacacggcccaaactcctacgggaggcagcagtagggaatcttccacaatggacgcaagtctgatggagcaacgccgcgtgagtgaagaaggttttcggatcgtaaagctctgttgttggtgaagaaggatagaggtagtaactggcctttatttgacggtaatcaaccagaaagtcacggctaactacgtgccagcagccgcggtaatacgtaggtggcaagcgttgtccggatttattgggcgtaaagcgagcgcaggcggaagaataagtctgatgtgaaagccctcggcttaaccgaggaactgcatcggaaactgtttttcttgagtgcagaagaggagagtggaactccatgtgtagcggtggaatgcgtagatatatggaagaacaccagtggcgaaggcggctctctggtctgcaactgacgctgaggctcgaaagcatgggtagcgaacaggattagataccctggtagtccatgccgtaaacgatgagtgctaagtgttgggaggtttccgcctctcagtgctgcagctaacgcattaagcactccgcctggggagtacgaccgcaaggttgaaactcaaaggaattgacgggggcccgcacaagcggtggagcatgtggtttaattcgaagcaacgcgaagaaccttaccaggtcttgacatctagtgccatttgtagagatacaaagttcccttcggggacgctaagacaggtggtgcatggctgtcgtcagctcgtgtcgtgagatgttgggttaagtcccgcaacgagcgcaacccttgttattagttgccagcattaagttgggcactctaatgagactgccggtgacaaaccggaggaaggtggggatgacgtcaagtcatcatgccccttatgacctgggctacacacgtgctacaatgggcagtacaacgagaagcgagcctgcgaaggcaagcggatctctgaaagctgttctcagttcggactgcagtctgcaactcgactgcacgaagctggaatcgctagtaatcgcggatcagcacgccgcggtgaatacgttcccgggccttgtacacaccgcccgtcacaccatgggagtctgcaatgcccaaagccggtggcctaaccttcgggaaggagccgt